European Patent Specification EP 3 559 206 B1, published December 3, 2025. Title: Methods for Producing Biomass Rich in DHA, Palmitic Acid and Protein Using a Eukaryotic Microorganism. Applicant: Mara Renewables Corporation. The sequence listing filed with the application follows.

SEQUENCE LISTING (19 sequences)

SEQ ID NO: 1 - DNA, 1770 bp, Artificial Sequence
  Synthetic Construct
  misc_feature (52)..(52): N is A or G
  misc_feature (118)..(118): N is A or T
  misc_feature (127)..(127): N is A or G
  misc_feature (128)..(128): N is C or T
  misc_feature (186)..(186): N is A or G
  misc_feature (255)..(255): N is A or T
  misc_feature (261)..(261): N is A, G or T
  misc_feature (453)..(453): N is A or G
  misc_feature (454)..(454): N is C or T
  misc_feature (496)..(496): N is A or G
  misc_feature (497)..(497): N is C or T
  misc_feature (557)..(557): N is A or G
  misc_feature (569)..(569): N is A or G
  misc_feature (655)..(655): N is A or T
  misc_feature (684)..(684): N is C or T
  misc_feature (687)..(687): N is A or T
  misc_feature (689)..(689): N is G or T
  misc_feature (690)..(690): N is C or T
  misc_feature (691)..(691): N is C or T
  misc_feature (692)..(692): N is A, G or T
  misc_feature (695)..(695): N is A or T
  misc_feature (697)..(697): N is A or T
  misc_feature (699)..(699): N is A or G
  misc_feature (700)..(700): N is G or T
  misc_feature (701)..(701): N is A or G
  misc_feature (702)..(702): N is A or T
  misc_feature (705)..(705): N is A or G
  misc_feature (802)..(802): N is C or T
  misc_feature (915)..(915): N is A or C
  misc_feature (925)..(925): N is C or T
  misc_feature (1000)..(1000): N is A or G
  misc_feature (1023)..(1023): N is A or T
  misc_feature (1026)..(1026): N is A, G, or T
  misc_feature (1043)..(1043): N is A or G
  misc_feature (1054)..(1054): N is A or G
  misc_feature (1104)..(1104): N is A or G
  misc_feature (1237)..(1237): N is A or G
  misc_feature (1248)..(1248): N is G or T
  misc_feature (1338)..(1338): N is A or G
  misc_feature (1345)..(1345): N is A or T
  misc_feature (1404)..(1404): N is C or T
  misc_feature (1421)..(1421): N is C or T
  misc_feature (1465)..(1465): N is A or G
  misc_feature (1469)..(1469): N is C or T
  misc_feature (1470)..(1470): N is C or T
  misc_feature (1472)..(1472): N is A or T
  misc_feature (1475)..(1475): N is A or T
  misc_feature (1476)..(1476): N is A or T
  misc_feature (1529)..(1529): N is C or T
  misc_feature (1546)..(1546): N is C or T
  misc_feature (1563)..(1563): N is A or G
  misc_feature (1630)..(1630): N is C or T
  misc_feature (1678)..(1678): N is A or T
  misc_feature (1681)..(1681): N is C or G
  misc_feature (1692)..(1692): N is A, C or G
  misc_feature (1699)..(1699): N is C or G
  misc_feature (1704)..(1704): N is G or T
caacctggttgatcctgccagtagtcatatgctcgtctcaaagattaagccntgcatgtgtaagtataagcgattgtactgtgagactgcgaacggctcattatatcagtaataattncttcggtannttcttttatatggatacctgcagtaattctggaaataatacatgctgtaagagccctntatggggctgcacttattagattgaagccgattttattggtgaatcatgataattgagcagattgactntttttngtcgatgaatcgtttgagtttctgccccatcagttgtcgacggtagtgtattggactacggtgactataacgggtgacggagagttagggctcgactccggagagggagcctgagagacggctaccatatccaaggatagcagcaggcgcgtaaattacccactgtggactccacgaggtagtgacgagaannatcgatgcgaagcgtgtatgcgttttgctatcggaatgagannaatgtaaaaccctcatcgaggatcaactggagggcaagtctggtgccagcagccgcggtnattccagctccngaagcatatgctaaagttgttgcagttaaaaagctcgtagttgaatttctggcatgggcgaccggtgctttccctgaatggggatngattgtctgtgttgccttggccatctttntcntnnnnttntngnnnnganatctttcactgtaatcaaagcagagtgttccaagcaggtcgtatgaccggtatgtttattatgggatgataagataggacttgggtgctattttgtnggtttgcacgcctgagtaatggttaataggaacagttgggggtattcgtatttaggagctagaggtgaaattcttggatttccgaaagacgaactagagcgaaggcatttacnaagcatgttntcattaatcaagaacgaaagtctggggatcgaagatgattagataccatcgtagtctagaccgtaaacgatgccnacttgcgattgttgggtgctttnttntatgggcctcagcagcngcacatgaganatcaaagtctttgggttccggggggagtatggtcgcaaggctgaaacttnaaggaattgacggaagggcaccaccaggagtggagcctgcggcttaatttgactcaacacgggaaaacttaccaggtccagacataggtaggattgacagattgagagctctttcatgattctatgggtggtngtgcatggccnttcttagttggtggagtgatttgtctggttaattccgttaacgaacgagacctcggcctactaaatagtgcgtggtatggcaacatagtncgttttnaacttcttagagggacatgtccggtttacgggcaggaagttcgaggcaataacaggtcngtgatgcccttagatgntctgggccgcacgcgcgctacactgatgggttcatcgggttttnattnnanttnntggaattgagtgcttggtcggaaggcctggctaatccttggaacgctcatcgngctggggctagattttngcaattattaatctccnacgaggaattcctagtaaacgcaagtcatcagcttgcattgaatacgtccctgccctttgtacacancgcccgtcgcacctaccgattgaacggtccgatgaaaccatgggatgnttntgtttggattnatttttngacanaggcagaactcgggtgaatcttattgtttagaggaaggtgaagtcgtaacaaggtttccgtagtga

SEQ ID NO: 2 - DNA, 23 bp, Artificial Sequence
  Synthetic Construct
caacctggttgatcctgccagta

SEQ ID NO: 3 - DNA, 24 bp, Artificial Sequence
  Synthetic Construct
tcactacggaaaccttgttacgac

SEQ ID NO: 4 - DNA, 17 bp, Artificial Sequence
  Synthetic Construct
caggaaacagctatgac

SEQ ID NO: 5 - DNA, 20 bp, Artificial Sequence
  Synthetic Construct
taatacgactcactataggg

SEQ ID NO: 6 - DNA, 20 bp, Artificial Sequence
  Synthetic Construct
gtctggtgccagcagccgcg

SEQ ID NO: 7 - DNA, 20 bp, Artificial Sequence
  Synthetic Construct
cttaaaggaattgacggaag

SEQ ID NO: 8 - DNA, 20 bp, Artificial Sequence
  Synthetic Construct
agctttttaactgcaacaac

SEQ ID NO: 9 - DNA, 18 bp, Artificial Sequence
  Synthetic Construct
ggccatgcaccaccaccc

SEQ ID NO: 10 - DNA, 1761 bp, Artificial Sequence
  Synthetic Construct
caacctggttgatcctgccagtagtcatatgctcgtctcaaagattaagccatgcatgtgtaagtataagcgattgtactgtgagactgcgaacggctcattatatcagtaataatttcttcggtagtttcttttatatggatacctgcagtaattctggaaataatacatgctgtaagagccctgtatggggctgcacttattagattgaagccgattttattggtgaatcatgataattgagcagattgactttttagtcgatgaatcgtttgagtttctgccccatcagttgtcgacggtagtgtattggactacggtgactataacgggtgacggagagttagggctcgactccggagagggagcctgagagacggctaccatatccaaggatagcagcaggcgcgtaaattacccactgtggactccacgaggtagtgacgagaaatatcgatgcgaagcgtgtatgcgttttgctatcggaatgagagcaatgtaaaaccctcatcgaggatcaactggagggcaagtctggtgccagcagccgcggtaattccagctccagaagcatatgctaaagttgttgcagttaaaaagctcgtagttgaatttctggcatgggcgaccggtgctttccctgaatggggattgattgtctgtgttgccttggccatctttttcttttctttattgatgagaaatctttcactgtaatcaaagcagagtgttccaagcaggtcgtatgaccggtatgtttattatgggatgataagataggacttgggtgctattttgttggtttgcacgcctgagtaatggttaataggaacagttgggggtattcgtatttaggagctagaggtgaaattcttggatttccgaaagacgaactagagcgaaggcatttaccaagcatgttttcattaatcaagaacgaaagtctggggatcgaagatgattagataccatcgtagtctagaccgtaaacgatgccaacttgcgattgttgggtgcttttttatgggcctcagcagcagcacatgagaaatcaaagtctttgggttccggggggagtatggtcgcaaggctgaaacttaaaggaattgacggaagggcaccaccaggagtggagcctgcggcttaatttgactcaacacgggaaaacttaccaggtccagacataggtaggattgacagattgagagctctttcatgattctatgggtggtggtgcatggccgttcttagttggtggagtgatttgtctggttaattccgttaacgaacgagacctcggcctactaaatagtgcgtggtatggcaacatagtacgttttaacttcttagagggacatgtccggtttacgggcaggaagttcgaggcaataacaggtctgtgatgcccttagatgctctgggccgcacgcgcgctacactgatgggttcatcgggttttaatttcattattggaattgagtgcttggtcggaaggcctggctaatccttggaacgctcatcgtgctggggctagatttttgcaattattaatctccaacgaggaattcctagtaaacgcaagtcatcagcttgcattgaatacgtccctgccctttgtacacaccgcccgtcgcacctaccgattgaacggtccgatgaaaccatgggatgtttgtgtttggattcatttttggacataggcagaactcgggtgaatcttattgtttagaggaaggtgaagtcgtaacaaggtttccgtag

SEQ ID NO: 11 - DNA, 1764 bp, Artificial Sequence
  Synthetic Construct
aacctggttgatcctgccagtagtcatatgctcgtctcaaagattaagccatgcatgtgtaagtataagcgattgtactgtgagactgcgaacggctcattatatcagtaataatttcttcggtagtttcttttatatggatacctgcagtaattctggaaataatacatgctgtaagagccctgtatggggctgcacttattagattgaagccgattttattggtgaatcatgataattgagcagattgactttttagtcgatgaatcgtttgagtttctgccccatcagttgtcgacggtagtgtattggactacggtgactataacgggtgacggagagttagggctcgactccggagagggagcctgagagacggctaccatatccaaggatagcagcaggcgcgtaaattacccactgtggactccacgaggtagtgacgagaaatatcgatgcgaagcgtgtatgcgttttgctatcggaatgagagcaatgtaaaaccctcatcgaggatcaactggagggcaagtctggtgccagcagccgcggtaattccagctccagaagcatatgctaaagttgttgcagttaaaaagctcgtagttgaatttctggcatgggcgaccggtgctttccctgaatggggatagattgtctgtgttgccttggccatctttttcttttctttttaggggagaaatctttcactgtaatcaaagcagagtgttccaagcaggtcgtatgaccggtatgtttattatgggatgataagataggacttgggtgctattttgtcggtttgcacgcctgagtaatggttaataggaacagttgggggtattcgtatttaggagctagaggtgaaattcttggatttccgaaagacgaactagagcgaaggcatttaccaagcatgttttcattaatcaagaacgaaagtctggggatcgaagatgattagataccatcgtagtctagaccgtaaacgatgccgacttgcgattgttgggtgcttttttatgggcctcagcagcagcacatgagaaatcaaagtctttgggttccggggggagtatggtcgcaaggctgaaacttaaaggaattgacggaagggcaccaccaggagtggagcctgcggcttaatttgactcaacacgggaaaacttaccaggtccagacataggtaggattgacagattgagagctctttcatgattctatgggtggtagtgcatggccgttcttagttggtggagtgatttgtctggttaattccgttaacgaacgagacctcggcctactaaatagtgcgtggtatggcaacatagtacgtttttacttcttagagggacatgtccggtttacgggcaggaagttcgaggcaataacaggtctgtgatgcccttagatgttctgggccgcacgcgcgctacactgatgggttcatcgggttttgattctattttatggaattgagtgcttggtcggaaggcctggctaatccttggaacgctcatcgtgctggggctagatttttgcaattattaatctccaacgaggaattcctagtaaacgcaagtcatcagcttgcattgaatacgtccctgccctttgtacacaccgcccgtcgcacctaccgattgaacggtccgatgaaaccatgggatgattctgtttggattaatttttggacagaggcagaactcgggtgaatcttattgtttagaggaaggtgaagtcgtaacaaggtttccgtagtga

SEQ ID NO: 12 - DNA, 1765 bp, Artificial Sequence
  Synthetic Construct
caacctggttgatcctgccagtagtcatatgctcgtctcaaagattaagccgtgcatgtgtaagtataagcgattgtactgtgagactgcgaacggctcattatatcagtaataatttcttcggtagcttcttttatatggatacctgcagtaattctggaaataatacatgctgtaagagccctgtatggggctgcacttattagattgaagccgattttattggtgaatcatgataattgagcagattgactatttttggtcgatgaatcgtttgagtttctgccccatcagttgtcgacggtagtgtattggactacggtgactataacgggtgacggagagttagggctcgactccggagagggagcctgagagacggctaccatatccaaggatagcagcaggcgcgtaaattacccactgtggactccacgaggtagtgacgagaaatatcgatgcgaagcgtgtatgcgttttgctatcggaatgagagcaatgtaaaaccctcatcgaggatcaactggagggcaagtctggtgccagcagccgcggtaattccagctccagaagcatatgctaaagttgttgcagttaaaaagctcgtagttgaatttctggcatgggcgaccggtgctttccctgaatggggattgattgtctgtgttgccttggccatctttctcatgctattttggtatgagatctttcactgtaatcaaagcagagtgttccaagcaggtcgtatgaccggtatgtttattatgggatgataagataggacttgggtgctattttgttggtttgcacgcctgagtaatggttaataggaacagttgggggtattcgtatttaggagctagaggtgaaattcttggatttccgaaagacgaactagagcgaaggcatttacaaagcatgttttcattaatcaagaacgaaagtctggggatcgaagatgattagataccatcgtagtctagaccgtaaacgatgccgacttgcgattgttgggtgctttttttatgggcctcagcagcggcacatgagaaatcaaagtctttgggttccggggggagtatggtcgcaaggctgaaacttgaaggaattgacggaagggcacaccaggagtggagcctgcggcttaatttgactcaacacgggaaaacttaccaggtccagacataggtaggattgacagattgagagctctttcatgattctatgggtggtggtgcatggccgttcttagttggtggagtgatttgtctggttaattccgttaacgaacgagacctcggcctactaaatagtgcgtggtatggcaacatagtacgttttaacttcttagagggacatgtccggtttacgggcaggaagttcgaggcaataacaggtctgtgatgcccttagatgttctgggccgcacgcgcgctacactgatgggttcatcgggttttaattctatttttggaattgagtgcttggtcggaaggcctggctaatccttggaacgctcatcgtgctggggctagatttttgcaattattaatctccaacgaggaattcctagtaaacgcaagtcatcagcttgcattgaatacgtccctgccctttgtacacatcgcccgtcgcacctaccgattgaacggtccgatgaaaccatgggatgtttgtgtttggattaatttttggacagaggcagaactcgggtgaatcttattgtttagaggaaggtgaagtcgtaacaaggtttccgtagtga

SEQ ID NO: 13 - DNA, 1767 bp, Artificial Sequence
  Synthetic Construct
caacctggttgatcctgccagtagtcatatgctcgtctcaaagattaagccatgcatgtgtaagtataagcgattgtactgtgagactgcgaacggctcattatatcagtaataatttcttcggtagtttcttttatatggatacctgcagtaattctggaaataatacatgctgtaagagccctgtatggggctgcacttattagattgaagccgattttattggtgaatcatgataattgagcagattgactatttttgtcgatgaatcgtttgagtttctgccccatcagttgtcgacggtagtgtattggactacggtgactataacgggtgacggagagttagggctcgactccggagagggagcctgagagacggctaccatatccaaggatagcagcaggcgcgtaaattacccactgtggactccacgaggtagtgacgagaagtatcgatgcgaagcgtgtatgcgttttgctatcggaatgagagcaatgtaaaaccctcatcgaggatcaactggagggcaagtctggtgccagcagccgcggtaattccagctccggaagcatatgctaaagttgttgcagttaaaaagctcgtagttgaatttctggcatgggcgaccggtgctttccctgaatggggatagattgtctgtgttgccttggccatctttttcttttctttattgatgagaaatctttcactgtaatcaaagcagagtgttccaagcaggtcgtatgaccggtatgtttattatgggatgataagataggacttgggtgctattttgttggtttgcacgcctgagtaatggttaataggaacagttgggggtattcgtatttaggagctagaggtgaaattcttggatttccgaaagacgaactagagcgaaggcatttaccaagcatgttctcattaatcaagaacgaaagtctggggatcgaagatgattagataccatcgtagtctagaccgtaaacgatgccgacttgcgattgttgggtgctttattatatgggcctcagcagcagcacatgagaaatcaaagtctttgggttccggggggagtatggtcgcaaggctgaaacttaaaggaattgacggaagggcaccaccaggagtggagcctgcggcttaatttgactcaacacgggaaaacttaccaggtccagacataggtaggattgacagattgagagctctttcatgattctatgggtggtggtgcatggcctttcttagttggtggagtgatttgtctggttaattccgttaacgaacgagacctcggcctactaaatagtgcgtggtatggcaacatagtgcgtttttacttcttagagggacatgtccggtttacgggcaggaagttcgaggcaataacaggtctgtgatgcccttagatgttctgggccgcacgcgcgctacactgatgggttcatcgggttttaatttcatttttggaattgagtgcttggtcggaaggcctggctaatccttggaacgctcatcgtgctggggctagattttcgcaattattaatctccaacgaggaattcctagtaaacgcaagtcatcagcttgcattgaatacgtccctgccctttgtacacaccgcccgtcgcacctaccgattgaacggtccgatgaaaccatgggatgtttctgtttggattgatttttcgacagaggcagaactcgggtgaatcttattgtttagaggaaggtgaagtcgtaacaaggtttccgtagtga

SEQ ID NO: 14 - DNA, 1761 bp, Artifcial Sequence; identical to SEQ ID NO: 10

SEQ ID NO: 15 - DNA, 1767 bp, Artificial Sequence
  Synthetic Construct
caacctggttgatccgccagtagtcatatgctcgtctcaaagattaagccatgcatgtgtaagtataagcgattgtactgtgagactgcgaacggctcattatatcagtaataatttcttcggtaatttcttttatatggatacctgcagtaattctggaaataatacatgctgtaagagccctgtatggggctgcacttattagattgaagccgattttattggtgaatcatgataattgagcagattgacttttttggtcgatgaatcgtttgagtttctgccccatcagttgtcgacggtagtgtattggactacggtgactataacgggtgacggagagttagggctcgactccggagagggagcctgagagacggctaccatatccaaggatagcagcaggcgcgtaaattacccactgtggactccacgaggtagtgacgagaaacatcgatgcgaagcgtgtatgcgttttgctatcggaatgagaacaatgtaaaaccctcatcgaggatcaactggagggcaagtctggtgccagcagccgcggtaattccagctccagaagcatatgctaaagttgttgcagttaaaaagctcgtagttgaatttctggcatgggcgaccggtgctttccctgaatggggattgattgtctgtgttgccttggccatctttctcatgctgttattggtatgagatctttcactgtaatcaaagcagagtgttccaagcaggtcgtatgaccggtatgtttattatgggatgataagataggacttgggtgctattttgttggtttgcacgcctgagtaatggttaataggaacagttgggggtattcgtatttaggagctagaggtgaaattcttggatttccgaaagacgaactagagcgaaggcatttaccaagcatgttttcattaatcaagaacgaaagtctggggatcgaagatgattagataccatcgtagtctagaccgtaaacgatgccgacttgcgattgttgggtgcttttttgtatgggcctcagcagcagcacatgagaaatcaaagtctttgggttccggggggagtatggtcgcaaggctgaaacttaaaggaattgacggaagggcaccaccaggagtggagcctgcggcttaatttgactcaacacgggaaaacttaccaggtccagacataggtaggattgacagattgagagctctttcatgattctatgggtggtggtgcatggccgttcttagttggtggagtgatttgtctggttaattccgttaacgaacgagacctcggcctactaaatagtgcgtggtatggcaacatagtacgttttaacttcttagagggacatgtccggtttacgggcaggaagttcgaggcaataacaggtctgtgatgcccttagatgttctgggccgcacgcgcgctacactgatgggttcatcgggttttaattctaatttttggaattgagtgcttggtcggaaggcctggctaatccttggaacgctcatcgcgctggggctagatttttgcaattattaatctccaacgaggaattcctagtaaacgcaagtcatcagcttgcattgaatacgtccctgccctttgtacacaccgcccgtcgcacctaccgattgaacggtccgatgaaaccatgggatgtttctgtttggattcatttttggacagaggcagaactcgggtgaatcttattgtttagaggaaggtgaagtcgtaacaaggtttccgtagtga

SEQ ID NO: 16 - DNA, 1765 bp, Artificial Sequence
  Synthetic Construct
caacctggttgatcctgccagtagtcatatgctcgtctcaaagattaagccatgcatgtgtaagtataagcgattgtactgtgagactgcgaacggctcattatatcagtaataatttcttcggtagtttcttttatatggatacctgcagtaattctggaaataatacatgctgtaagagccctatatggggctgcacttattagattgaagccgattttattggtgaatcatgataattgagcagattgactttttagtcgatgaatcgtttgagtttctgccccatcagttgtcgacggtagtgtattggactacggtgactataacgggtgacggagagttagggctcgactccggagagggagcctgagagacggctaccatatccaaggatagcagcaggcgcgtaaattacccactgtggactccacgaggtagtgacgagaaatatcgatgcgaagcgtgtatgcgttttgctatcggaatgagagcaatgtaaaaccctcatcgaggatcaactggagggcaagtctggtgccagcagccgcggtaattccagctccagaagcatatgctaaagttgttgcagttaaaaagctcgtagttgaatttctggcatgggcgaccggtgctttccctgaatggggattgattgtctgtgttgccttggccatctttttcttttctttttaggggagaaatctttcactgtaatcaaagcagagtgttccaagcaggtcgtatgaccggtatgtttattatgggatgataagataggacttgggtgctattttgttggtttgcacgcctgagtaatggttaataggaacagttgggggtattcgtatttaggagctagaggtgaaattcttggatttccgaaagacgaactagagcgaaggcatttaccaagcatgttttcattaatcaagaacgaaagtctggggatcgaagatgattagataccatcgtagtctagaccgtaaacgatgccgacttgcgattgttgggtgcttttttatgggcctcagcagcagcacatgagagatcaaagtctttgggttccggggggagtatggtcgcaaggctgaaacttaaaggaattgacggaagggcaccaccaggagtggagcctgcggcttaatttgactcaacacgggaaaacttaccaggtccagacataggtaggattgacagattgagagctctttcatgattctatgggtggtggtgcatggccgttcttagttggtggagtgatttgtctggttaattccgttaacgaacgagacctcggcctactaaatagtgcgtggtatggcaacatagtacgtttttacttcttagagggacatgtccggtttacgggcaggaagttcgaggcaataacaggtccgtgatgcccttagatgttctgggccgcacgcgcgctacactgatgggttcatcgggttttgattctattttatggaattgagtgcttggtcggaaggcctggctaatccttggaacgctcatcgtgctggggctagatttttgcaattattaatctccaacgaggaattcctagtaaacgcaagtcatcagcttgcattgaatacgtccctgccctttgtacacaccgcccgtcgcacctaccgattgaacggtccgatgaaaccatgggatgtttctgtttggattaatttttggacagaggcagaactcgggtgaatcttattgtttagaggaaggtgaagtcgtaacaaggtttccgtagtga

SEQ ID NO: 17 - DNA, 1765 bp, Artificial Sequence; identical to SEQ ID NO: 16
  Synthetic Construct

SEQ ID NO: 18 - DNA, 1767 bp, Artificial Sequence
  Synthetic Construct
caacctggttgatcctgccagtagtcatatgctcgtctcaaagattaagccatgcatgtgtaagtataagcgattgtactgtgagactgcgaacggctcattatatcagtaataatttcttcggtagtttcttttatatggatacctgcagtaattctggaaataatacatgctgtaagagccctgtatggggctgcacttattagattgaagccgattttattggtgaatcatgataattgagcagattgactattttggtcgatgaatcgtttgagtttctgccccatcagttgtcgacggtagtgtattggactacggtgactataacgggtgacggagagttagggctcgactccggagagggagcctgagagacggctaccatatccaaggatagcagcaggcgcgtaaattacccactgtggactccacgaggtagtgacgagaaatatcgatgcgaagcgtgtatgcgttttgctatcggaatgagagtaatgtaaaaccctcatcgaggatcaactggagggcaagtctggtgccagcagccgcggtaattccagctccagaagcatatgctaaagttgttgcagttaaaaagctcgtagttgaatttctggcatgggcgaccggtgctttccctgaatggggattgattgtctgtgttgccttggccatctttttcttttctttattggggagaaatctttcactgtaatcaaagcagagtgttccaagcaggtcgtatgaccggtatgtttattatgggatgataagataggacttgggtgctattttgttggtttgcacgcctgagtaatggttaataggaacagttgggggtattcgtatttaggagctagaggtgaaattcttggatttccgaaagacgaactagagcgaaggcatttaccaagcatgttttcattaatcaagaacgaaagtctggggatcgaagatgattagataccatcgtagtctagaccgtaaacgatgccgacttgcgattgttgggtgcttttttatgggcctcagcagcagcacatgagaaatcaaagtctttgggttccggggggagtatggtcgcaaggctgaaacttaaaggaattgacggaagggcaccaccaggagtggagcctgcggcttaatttgactcaacacgggaaaacttaccaggtccagacataggtaggattgacagattgagagctctttcatgattctatgggtggtggtgcatggccgttcttagttggtggagtgatttgtctggttaattccgttaacgaacgagacctcggcctactaaatagtgcgtggtatggcaacatagtgcgtttttaacttcttagagggacatgtccggtttacgggcaggaagttcgaggcaataacaggtctgtgatgcccttagatgttctgggccgcacgcgcgctacactgatgggttcatcgggttttaatttcatttaatggaattgagtgcttggtcggaaggcctggctaatccttggaacgctcatcgtgctggggctagatttttgcaattattaatctccaacgaggaattcctagtaaacgcaagtcatcagcttgcattgaatacgtccctgccctttgtacacaccgcccgtcgcacctaccgattgaacggtccgatgaaaccatgggatgtttgtgtttggattaatttttggacataggcagaactcgggtgaatcttattgtttagaggaaggtgaagtcgtaacaaggtttccgtagtga

SEQ ID NO: 19 - DNA, 1769 bp, Artificial Sequence
  Synthetic Construct
caacctggttgatcctgccagtagtcatatgctcgtctcaaagattaagccatgcatgtgtaagtataagcgattgtactgtgagactgcgaacggctcattatatcagtaataattacttcggtagtttcttttatatggatacctgcagtaattctggaaataatacatgctgtaagagccctgtatggggctgcacttattagattgaagccgattttattggtgaatcatgataattgagcagattgactatttttggtcgatgaatcgtttgagtttctgccccatcagttgtcgacggtagtgtattggactacggtgactataacgggtgacggagagttagggctcgactccggagagggagcctgagagacggctaccatatccaaggatagcagcaggcgcgtaaattacccactgtggactccacgaggtagtgacgagaaatatcgatgcgaagcgtgtatgcgttttgctatcggaatgagagcaatgtaaaaccctcatcgaggatcaactggagggcaagtctggtgccagcagccgcggtgattccagctccagaagcatatgctaaagttgttgcagttaaaaagctcgtagttgaatttctggcatgggcgaccggtgctttccctgaatggggattgattgtctgtgttgccttggccatctttttcttttctttattggggagaaatctttcactgtaatcaaagcagagtgttccaagcaggtcgtatgaccggtatgtttattatgggatgataagataggacttgggtgctattttgttggtttgcacgcctgagtaatggttaataggaacagttgggggtattcgtatttaggagctagaggtgaaattcttggatttccgaaagacgaactagagcgaaggcatttaccaagcatgttttcattaatcaagaacgaaagtctggggatcgaagatgattagataccatcgtagtctagaccgtaaacgatgccgacttgcgattgttgggtgcttttttttatgggcctcagcagcagcacatgagaaatcaaagtctttgggttccggggggagtatggtcgcaaggctgaaacttaaaggaattgacggaagggcaccaccaggagtggagcctgcggcttaatttgactcaacacgggaaaacttaccaggtccagacataggtaggattgacagattgagagctctttcatgattctatgggtggtggtgcatggccgttcttagttggtggagtgatttgtctggttaattccgttaacgaacgagacctcggcctactaaatagtgcgtggtatggcaacatagtacgtttttacttcttagagggacatgtccggtttacgggcaggaagttcgaggcaataacaggtctgtgatgcccttagatgttctgggccgcacgcgcgctacactgatgggttcatcgggttttaatttcaatttttggaattgagtgcttggtcggaaggcctggctaatccttggaacgctcatcgtgctggggctagatttttgcaattattaatctccgacgaggaattcctagtaaacgcaagtcatcagcttgcattgaatacgtccctgccctttgtacacaccgcccgtcgcacctaccgattgaacggtccgatgaaaccatgggatgtttctgtttggattcatttttggacagaggcagaactcgggtgaatcttattgtttagaggaaggtgaagtcgtaacaaggtttccgtagtga